European Patent Specification EP 3 509 576 B1, published October 30, 2024. Title: Compositions and Methods for Regulating Melanogenesis. Applicant: Agency for Science, Technology and Research. The sequence listing filed with the application follows.

SEQUENCE LISTING (8 sequences)

SEQ ID NO: 1 - DNA, 21 bp, Artificial Sequence
  TYR forward primer
tgcacagagagacgactcttg

SEQ ID NO: 2 - DNA, 21 bp, Artificial Sequence
  TYR reverse primer
ggcatggactgtggtcatgag

SEQ ID NO: 3 - DNA, 22 bp, Artificial Sequence
  TYRP1 forward primer
tctctgggctgtatcttcttcc

SEQ ID NO: 4 - DNA, 21 bp, Artificial Sequence
  TYRP1 reverse primer
gtctgggcaacacataccact

SEQ ID NO: 5 - DNA, 20 bp, Artificial Sequence
  DCT forward primer
cttgggctgcaaaatcctgc

SEQ ID NO: 6 - DNA, 21 bp, Artificial Sequence
  DCT reverse primer
cagcactccttgttcactagg

SEQ ID NO: 7 - DNA, 23 bp, Artificial Sequence
  PMEL forward primer
agtgcctactacagaagttgtgg

SEQ ID NO: 8 - DNA, 21 bp, Artificial Sequence
  PMEL reverse primer
cacaggtgcagtgcttatgac